European Patent Application EP 4 144 748 A1, published March 8, 2023. Title: HUMAN INTERFERON-BETA VARIANT WITH DOUBLE MUTATION AND METHOD FOR IMPROVING STABILITY OF HUMAN INTERFERON-BETA VARIANT. Applicant: Abion Inc. Application EP21796576.3. The sequence listing filed with the application follows.

SEQUENCE LISTING (5 sequences)

SEQ ID NO: 1 - protein, 166 aa, Artificial Sequence
  Human interferon beta protein
MSYNLLGFLQRSSNFQCQKLLWQLNGRLEYCLKDRMNFDIPEEIKQLQQFQKEDAALTIYEMLQNIFAIFRQDSSSTGWNETIVENLLANVYHQINHLKTVLEEKLEKEDFTRGKLMSSLHLKRYYGRILHYLKAKEYSHCAWTIVRVEILRNFYFINRLTGYLRN

SEQ ID NO: 2 - protein, 166 aa, Artificial Sequence
  Human interferon beta R27T mutein (ABN101(NT))
MSYNLLGFLQRSSNFQCQKLLWQLNGTLEYCLKDRMNFDIPEEIKQLQQFQKEDAALTIYEMLQNIFAIFRQDSSSTGWNETIVENLLANVYHQINHLKTVLEEKLEKEDFTRGKLMSSLHLKRYYGRILHYLKAKEYSHCAWTIVRVEILRNFYFINRLTGYLRN

SEQ ID NO: 3 - protein, 166 aa, Artificial Sequence
  Human interferon beta R27T, C17S double mutein (ABN101(CS))
MSYNLLGFLQRSSNFQSQKLLWQLNGTLEYCLKDRMNFDIPEEIKQLQQFQKEDAALTIYEMLQNIFAIFRQDSSSTGWNETIVENLLANVYHQINHLKTVLEEKLEKEDFTRGKLMSSLHLKRYYGRILHYLKAKEYSHCAWTIVRVEILRNFYFINRLTGYLRN

SEQ ID NO: 4 - DNA, 21 bp, Artificial Sequence
  Xba1 forward primer
ggtctagagccaccatgacca

SEQ ID NO: 5 - DNA, 34 bp, Artificial Sequence
  Pac1 reverse prier
cacttagggattaattaatcagttcctcaggtag